European Patent Specification EP 3 895 736 B1, published April 19, 2023. Title: Antibody-drug conjugates targeting uPARAP. Applicant: Rigshospitalet University of Copenhagen. The sequence listing filed with the application follows.

SEQUENCE LISTING (59 sequences)

SEQ ID NO: 1 - protein, 214 aa, Mus musculus
DIQMTQSPASQSASLGESVTITCLASQTIGTWLAWYQQKPGKSPQLLIYAATTLTDGVPSRFSGAGSGTKFSLKISSLQAEDFASYFCQEFFSTPFTFGSGTKLELKRADAAPTVSIFPPSSEQLTSGGASVVCFLNNFYPKDINVKWKIDGGERQNGVLNSWTDQDSKDSTYSMSSTLTLTKDEYERHNSYTCEATHKTSTSPIVKSFNRNEC

SEQ ID NO: 2 - protein, 11 aa, Mus musculus
LASQTIGTWLA

SEQ ID NO: 3 - protein, 7 aa, Mus musculus
AATTLTD

SEQ ID NO: 4 - protein, 9 aa, Mus musculus
QEFFSTPFT

SEQ ID NO: 5 - protein, 446 aa, Mus musculus
QVQLQQPGTELVRPGLSVKLSCKASGYTFTSYWMNWVKQRPGQGLEWIGMIHPSNDEKRINQKFKDKATLTVDKFSSTVYMQVSSPTSEDSAVYYCARGGGDYVGDYALDFWGQGTSVTVSSAKTTPPSVYPLAPGSAAQTNSMVTLGCLVKGYFPEPVTVTWNSGSLSSGVHTFPAVLQSDLYTLSSSVTVPSSTWPSETVTCNVAHPASSTKVDKKIVPRDCGCKPCICTVPEVSSVFIFPPKPKDVLTITLTPKVTCVVVDISKDDPEVQFSWFVDDVEVHTAQTQPREEQFNSTFRSVSELPIMHQDWLNGKEFKCRVNSAAFPAPIEKTISKTKGRPKAPQVYTIPPPKEQMAKDKVSLTCMITDFFPEDITVEWQWNGQPAENYKNTQPIMDTDGSYFIYSKLNVQKSNWEAGNTFTCSVLHEGLHNHHTEKSLSHSPGK

SEQ ID NO: 6 - protein, 5 aa, Mus musculus
SYWMN

SEQ ID NO: 7 - protein, 17 aa, Mus musculus
MIHPSNDEKRINQKFKD

SEQ ID NO: 8 - protein, 13 aa, Mus musculus
GGGDYVGDYALDF

SEQ ID NO: 9 - protein, 214 aa, Mus musculus
DIQMTQSPASQSASLGESVTITCLASQTIGTWLAWYQQKPGKSPQLLIYAATTLTDGVPSRFSGAGSGTKFSLKISSLQAEDFASYFCQEFFSTPFTFGSGTKLELKRADAAPTVSIFPPSSEQLTSGGASVVCFLNNFYPKDINVKWKIDGSERQNGVLNSWTDQDSKDSTYSMSSTLTLTKDEYERHNSYTCEATHKTSTSPIVKSFNRNEC

SEQ ID NO: 10 - protein, 224 aa, Mus musculus
QVQLQQPGTELVRPGLSVKLSCKASGYTFTSYWMNWVKQRPGQGLEWIGMIHPSNDEKRINQKFKDKATLTVDKFSSTVYMQVSSPTSEDSAVYYCARGGGDYVGDYALDFWGQGTSVTVSSAKTTPPSVYPLAPGSAAQTNSMVTLGCLVKGYFPEPVTVTWNSGSLSSGVHTFPAVLQSDLYTLSSSVTVPSSTWPSETVTCNVAHPASSTKVDKKIVPRDC

SEQ ID NO: 11 - protein, 107 aa, Mus musculus
DIVMTQSQKFMSTSLGARVSITCKASQNVGSNVVWYQQKLGQSPKALIYSASSRFSGVPDRFTGSGSGTDFTLTISNVQSEDLAEYFCQQYNTYPLAFGAGTKLELK

SEQ ID NO: 12 - protein, 11 aa, Mus musculus
KASQNVGSNVV

SEQ ID NO: 13 - protein, 7 aa, Mus musculus
SASSRFS

SEQ ID NO: 14 - protein, 9 aa, Mus musculus
QQYNTYPLA

SEQ ID NO: 15 - protein, 119 aa, Mus musculus
DVQLQESGPGLVKPSQSLSVTCTVTGYSITNAYYWNWIRHFPGNKLEWLGYIHSSGDTNYNPSLKSRISITRDTSKNQFFLQLNSVTTEDTATYYCARSPYYSNYFPYWGQGTLVTVSA

SEQ ID NO: 16 - protein, 6 aa, Mus musculus
NAYYWN

SEQ ID NO: 17 - protein, 16 aa, Mus musculus
YIHSSGDTNYNPSLKS

SEQ ID NO: 18 - protein, 10 aa, Mus musculus
SPYYSNYFPY

SEQ ID NO: 19 - protein, 214 aa, Mus musculus
  MISC_FEATURE (1)..(7): subject to potential ambiguity due to the position of primer regions in the sequence determination
DILMTQSQKFMSTSVGDRVSVTCKASQNVDTYVVWYQQKPGQSPKPLIYSASSRFSGVPDRFTGTGSGTDFTLTINNVQSEDLAEYFCQQYHNSPLTFGGGTKLEIKRADAAPTVSIFPPSSEQLTSGGASVVCFLNNFYPKDINVKWKIDGSERQNGVLNSWTDQDSKDSTYSMSSTLTLTKDEYERHNSYTCEATHKTSTSPIVKSFNRNEC

SEQ ID NO: 20 - protein, 207 aa, Mus musculus
QKFMSTSVGDRVSVTCKASQNVDTYVVWYQQKPGQSPKPLIYSASSRFSGVPDRFTGTGSGTDFTLTINNVQSEDLAEYFCQQYHNSPLTFGGGTKLEIKRADAAPTVSIFPPSSEQLTSGGASVVCFLNNFYPKDINVKWKIDGSERQNGVLNSWTDQDSKDSTYSMSSTLTLTKDEYERHNSYTCEATHKTSTSPIVKSFNRNEC

SEQ ID NO: 21 - protein, 11 aa, Mus musculus
KASQNVDTYVV

SEQ ID NO: 22 - protein, 7 aa, Mus musculus
SASSRFS

SEQ ID NO: 23 - protein, 9 aa, Mus musculus
QQYHNSPLT

SEQ ID NO: 24 - protein, 221 aa, Mus musculus
  MISC_FEATURE (1)..(8): subject to potential ambiguity due to the position of primer regions in the sequence determination
QVHLQQSGPELKKPGETVKISCKASGYIFIDYGMHWVKQAPGKGLKWMGSINTKSGVSTYAAEFKGRFAFSLETSASTAYLQINNLKNEDTATYFCARPPYYSQYGSYWGQGTLVTVSAAKTTPPSVYPLAPGSAAQTNSMVTLGCLVKGYFPEPVTVTWNSGSLSSGVHTFPAVLQSDLYTLSSSVTVPSSTWPSETVTCNVAHPASSTKVDKKIVPRDC

SEQ ID NO: 25 - protein, 213 aa, Mus musculus
PELKKPGETVKISCKASGYIFIDYGMHWVKQAPGKGLKWMGSINTKSGVSTYAAEFKGRFAFSLETSASTAYLQINNLKNEDTATYFCARPPYYSQYGSYWGQGTLVTVSAAKTTPPSVYPLAPGSAAQTNSMVTLGCLVKGYFPEPVTVTWNSGSLSSGVHTFPAVLQSDLYTLSSSVTVPSSTWPSETVTCNVAHPASSTKVDKKIVPRDC

SEQ ID NO: 26 - protein, 5 aa, Mus musculus
DYGMH

SEQ ID NO: 27 - protein, 17 aa, Mus musculus
SINTKSGVSTYAAEFKG

SEQ ID NO: 28 - protein, 10 aa, Mus musculus
PPYYSQYGSY

SEQ ID NO: 29 - protein, 1479 aa, Homo sapiens
MGPGRPAPAPWPRHLLRCVLLLGCLHLGRPGAPGDAALPEPNVFLIFSHGLQGCLEAQGGQVRVTPACNTSLPAQRWKWVSRNRLFNLGTMQCLGTGWPGTNTTASLGMYECDREALNLRWHCRTLGDQLSLLLGARTSNISKPGTLERGDQTRSGQWRIYGSEEDLCALPYHEVYTIQGNSHGKPCTIPFKYDNQWFHGCTSTGREDGHLWCATTQDYGKDERWGFCPIKSNDCETFWDKDQLTDSCYQFNFQSTLSWREAWASCEQQGADLLSITEIHEQTYINGLLTGYSSTLWIGLNDLDTSGGWQWSDNSPLKYLNWESDQPDNPSEENCGVIRTESSGGWQNRDCSIALPYVCKKKPNATAEPTPPDRWANVKVECEPSWQPFQGHCYRLQAEKRSWQESKKACLRGGGDLVSIHSMAELEFITKQIKQEVEELWIGLNDLKLQMNFEWSDGSLVSFTHWHPFEPNNFRDSLEDCVTIWGPEGRWNDSPCNQSLPSICKKAGQLSQGAAEEDHGCRKGWTWHSPSCYWLGEDQVTYSEARRLCTDHGSQLVTITNRFEQAFVSSLIYNWEGEYFWTALQDLNSTGSFFWLSGDEVMYTHWNRDQPGYSRGGCVALATGSAMGLWEVKNCTSFRARYICRQSLGTPVTPELPGPDPTPSLTGSCPQGWASDTKLRYCYKVFSSERLQDKKSWVQAQGACQELGAQLLSLASYEEEHFVANMLNKIFGESEPEIHEQHWFWIGLNRRDPRGGQSWRWSDGVGFSYHNFDRSRHDDDDIRGCAVLDLASLQWVAMQCDTQLDWICKIPRGTDVREPDDSPQGRREWLRFQEAEYKFFEHHSTWAQAQRICTWFQAELTSVHSQAELDFLSHNLQKFSRAQEQHWWIGLHTSESDGRFRWTDGSIINFISWAPGKPRPVGKDKKCVYMTASREDWGDQRCLTALPYICKRSNVTKETQPPDLPTTALGGCPSDWIQFLNKCFQVQGQEPQSRVKWSEAQFSCEQQEAQLVTITNPLEQAFITASLPNVTFDLWIGLHASQRDFQWVEQEPLMYANWAPGEPSGPSPAPSGNKPTSCAVVLHSPSAHFTGRWDDRSCTEETHGFICQKGTDPSLSPSPAALPPAPGTELSYLNGTFRLLQKPLRWHDALLLCESHNASLAYVPDPYTQAFLTQAARGLRTPLWIGLAGEEGSRRYSWVSEEPLNYVGWQDGEPQQPGGCTYVDVDGAWRTTSCDTKLQGAVCGVSSGPPPPRRISYHGSCPQGLADSAWIPFREHCYSFHMELLLGHKEARQRCQRAGGAVLSILDEMENVFVWEHLQSYEGQSRGAWLGMNFNPKGGTLVWQDNTAVNYSNWGPPGLGPSMLSHNSCYWIQSNSGLWRPGACTNITMGVVCKLPRAEQSSFSPSALPENPAALVVVLMAVLLLLALLTAALILYRRRQSIERGAFEGARYSRSSSSPTEATEKNILVSDMEMNEQQE

SEQ ID NO: 30 - protein, 116 aa, Homo sapiens
IFSHGLQGCLEAQGGQVRVTPACNTSLPAQRWKWVSRNRLFNLGTMQCLGTGWPGTNTTASLGMYECDREALNLRWHCRTLGDQLSLLLGARTSNISKPGTLERGDQTRSGQWRIY

SEQ ID NO: 31 - protein, 121 aa, Homo sapiens
PNVFLIFSHGLQGCLEAQGGQVRVTPACNTSLPAQRWKWVSRNRLFNLGTMQCLGTGWPGTNTTASLGMYECDREALNLRWHCRTLGDQLSLLLGARTSNISKPGTLERGDQTRSGQWRIY

SEQ ID NO: 32 - protein, 48 aa, Homo sapiens
NSHGKPCTIPFKYDNQWFHGCTSTGREDGHLWCATTQDYGKDERWGFC

SEQ ID NO: 33 - protein, 49 aa, Homo sapiens
GNSHGKPCTIPFKYDNQWFHGCTSTGREDGHLWCATTQDYGKDERWGFC

SEQ ID NO: 34 - protein, 115 aa, Homo sapiens
SCYQFNFQSTLSWREAWASCEQQGADLLSITEIHEQTYINGLLTGYSSTLWIGLNDLDTSGGWQWSDNSPLKYLNWESDQPDNPSEENCGVIRTESSGGWQNRDCSIALPYVCKK

SEQ ID NO: 35 - protein, 126 aa, Homo sapiens
CETFWDKDQLTDSCYQFNFQSTLSWREAWASCEQQGADLLSITEIHEQTYINGLLTGYSSTLWIGLNDLDTSGGWQWSDNSPLKYLNWESDQPDNPSEENCGVIRTESSGGWQNRDCSIALPYVCK

SEQ ID NO: 36 - protein, 316 aa, Homo sapiens
IFSHGLQGCLEAQGGQVRVTPACNTSLPAQRWKWVSRNRLFNLGTMQCLGTGWPGTNTTASLGMYECDREALNLRWHCRTLGDQLSLLLGARTSNISKPGTLERGDQTRSGQWRIYGSEEDLCALPYHEVYTIQGNSHGKPCTIPFKYDNQWFHGCTSTGREDGHLWCATTQDYGKDERWGFCPIKSNDCETFWDKDQLTDSCYQFNFQSTLSWREAWASCEQQGADLLSITEIHEQTYINGLLTGYSSTLWIGLNDLDTSGGWQWSDNSPLKYLNWESDQPDNPSEENCGVIRTESSGGWQNRDCSIALPYVCKK

SEQ ID NO: 37 - protein, 320 aa, Homo sapiens
PNVFLIFSHGLQGCLEAQGGQVRVTPACNTSLPAQRWKWVSRNRLFNLGTMQCLGTGWPGTNTTASLGMYECDREALNLRWHCRTLGDQLSLLLGARTSNISKPGTLERGDQTRSGQWRIYGSEEDLCALPYHEVYTIQGNSHGKPCTIPFKYDNQWFHGCTSTGREDGHLWCATTQDYGKDERWGFCPIKSNDCETFWDKDQLTDSCYQFNFQSTLSWREAWASCEQQGADLLSITEIHEQTYINGLLTGYSSTLWIGLNDLDTSGGWQWSDNSPLKYLNWESDQPDNPSEENCGVIRTESSGGWQNRDCSIALPYVCK

SEQ ID NO: 38 - protein, 183 aa, Homo sapiens
IFSHGLQGCLEAQGGQVRVTPACNTSLPAQRWKWVSRNRLFNLGTMQCLGTGWPGTNTTASLGMYECDREALNLRWHCRTLGDQLSLLLGARTSNISKPGTLERGDQTRSGQWRIYGSEEDLCALPYHEVYTIQGNSHGKPCTIPFKYDNQWFHGCTSTGREDGHLWCATTQDYGKDERWGFC

SEQ ID NO: 39 - protein, 188 aa, Homo sapiens
PNVFLIFSHGLQGCLEAQGGQVRVTPACNTSLPAQRWKWVSRNRLFNLGTMQCLGTGWPGTNTTASLGMYECDREALNLRWHCRTLGDQLSLLLGARTSNISKPGTLERGDQTRSGQWRIYGSEEDLCALPYHEVYTIQGNSHGKPCTIPFKYDNQWFHGCTSTGREDGHLWCATTQDYGKDERWGFC

SEQ ID NO: 40 - protein, 181 aa, Homo sapiens
NSHGKPCTIPFKYDNQWFHGCTSTGREDGHLWCATTQDYGKDERWGFCPIKSNDCETFWDKDQLTDSCYQFNFQSTLSWREAWASCEQQGADLLSITEIHEQTYINGLLTGYSSTLWIGLNDLDTSGGWQWSDNSPLKYLNWESDQPDNPSEENCGVIRTESSGGWQNRDCSIALPYVCKK

SEQ ID NO: 41 - protein, 181 aa, Homo sapiens
GNSHGKPCTIPFKYDNQWFHGCTSTGREDGHLWCATTQDYGKDERWGFCPIKSNDCETFWDKDQLTDSCYQFNFQSTLSWREAWASCEQQGADLLSITEIHEQTYINGLLTGYSSTLWIGLNDLDTSGGWQWSDNSPLKYLNWESDQPDNPSEENCGVIRTESSGGWQNRDCSIALPYVCK

SEQ ID NO: 42 - protein, 8 aa, Mus musculus
QTIGTWLA

SEQ ID NO: 43 - protein, 11 aa, Mus musculus
LLIYAATTLTD

SEQ ID NO: 44 - protein, 8 aa, Mus musculus
QEFFSTPF

SEQ ID NO: 45 - protein, 9 aa, Mus musculus
YTFTSYWMN

SEQ ID NO: 46 - protein, 14 aa, Mus musculus
WIGMIHPSNDEKRI

SEQ ID NO: 47 - protein, 14 aa, Mus musculus
RGGGDYVGDYALDF

SEQ ID NO: 48 - protein, 8 aa, Mus musculus
QNVGSNVV

SEQ ID NO: 49 - protein, 11 aa, Mus musculus
ALIYSASSRFS

SEQ ID NO: 50 - protein, 9 aa, Mus musculus
QQYNTYPLA

SEQ ID NO: 51 - protein, 10 aa, Mus musculus
YSITNAYYWN

SEQ ID NO: 52 - protein, 13 aa, Mus musculus
WLGYIHSSGDTNY

SEQ ID NO: 53 - protein, 11 aa, Mus musculus
RSPYYSNYFPY

SEQ ID NO: 54 - protein, 8 aa, Mus musculus
QNVDTYVV

SEQ ID NO: 55 - protein, 11 aa, Mus musculus
PLIYSASSRFS

SEQ ID NO: 56 - protein, 8 aa, Mus musculus
QQYHNSPL

SEQ ID NO: 57 - protein, 9 aa, Mus musculus
YIFIDYGMH

SEQ ID NO: 58 - protein, 14 aa, Mus musculus
WMGSINTKSGVSTY

SEQ ID NO: 59 - protein, 11 aa, Mus musculus
RPPYYSQYGSY